European Patent Specification EP 3 607 038 B1, published May 6, 2026. Title: CLEANING COMPOSITIONS AND USES THEREOF. Applicant: Novozymes A/S. The sequence listing filed with the application follows.

SEQUENCE LISTING (86 sequences)

SEQ ID NO: 1 - protein, 182 aa, Bacillus sp-62451
LPPDLPSKSTTQAQLNSLNVKNEESMSGYSREKFPHWISQGDGCDTRQVILKRDADNYSGNCPVTSGKWYSYYDGITFNDPSQLDIDHVVPLAEAWRSGASSWSTAKREDFANDLNGPQLIAVSASSNRSKGDQDPSTWQPPRAGANCAYAKMWINTKYNWGLHLQSSEKTALQGMLNSCSY

SEQ ID NO: 2 - protein, 182 aa, Bacillus horikoshii
LPPGTPTKSEAQNQLNSLTVKSEGSMTGYSRDLFPHWSGQGNGCDTRQIVLQRDADYYTGTCPTTSGKWYSYFDGVIVYSPSEIDIDHIVPLAEAWRSGASSWTTEQRRAFANDLNGPQLIAVTASVNRSKGDQDPSTWQPPRAGARCAYAKWWINTKHRWNLHLQSSEKSSLQTMLNGCAY

SEQ ID NO: 3 - protein, 182 aa, Bacillus sp-62520
LPPGTPSKSEAQSQLNALTVKPEDPMTGYSRDHFPHWISQGNGCNTRQIVLQRDADYYSGACPVTTGKWYSYFDGVIVYSPSEIDIDHIVPLAEAWRSGASSWTTEKRRSFANDLNGPQLIAVTASVNRSKGDQDPSTWQPPRAGARCAYAKWWINTKHRWGLHLQSSEKSSLQSMLNGCAY

SEQ ID NO: 4 - protein, 182 aa, Bacillus sp-62520
LPPGTPSKSEAQSQLNALTVKPEDPMTGYSRDHFPHWISQGNGCNTRQIVLQRDADYYSGACPVTTGKWYSYFDGVIVYSPSEIDIDHIVPLAEAWRSGASSWTTEQRRSFANDLNGPQLIAVTASVNRSKGDQDPSTWQPPRAGARCAYAKWWINTKHRWGLHLQSSEKSSLQSMLNGCAY

SEQ ID NO: 5 - protein, 182 aa, Bacillus horikoshii
LPPGTPSKSEAQSQLNSLTVKSEDPMTGYSRDHFPHWSGQGNGCDTRQIVLQRDADYYSGNCPVTSGKWYSYFDGVIVYSPSEIDIDHVVPLAEAWRSGASSWTTEQRRSFANDLNGPQLIAVTASVNRSKGDQDPSTWQPPRAGARCAYAKWWINTKHRWNLHLQSSEKSALQTMLNGCVY

SEQ ID NO: 6 - protein, 182 aa, Bacillus horikoshii
LPPGTPSKSEAQSQLNSLTVKTEDPMTGYSRDLFPHWSGQGSGCDTRQIVLQRDADYFTGTCPTTSGKWYSYFDGVIVYSPSEIDVDHIVPLAEAWRSGASSWTTEQRRAFANDLTGPQLIAVTASVNRSKGDQDPSTWQPPRAGARCAYAKWWINTKHRWNLHLQSSEKSSLQTMLNGCAY

SEQ ID NO: 7 - protein, 182 aa, Bacillus sp-16840
LPPGTPSKSEAQSQLNALTVKAEDPMTGYSRNLFPHWNSQGNGCNTRQLVLQRDADYYSGNCPVTSGRWYSYFDGVVVTSPSEIDIDHIVPLAEAWRSGASSWTTEKRKEFANDLNGPQLIAVTASVNRSKGDQDPSTWQPPRAAARCGYAKWWINTKYRWDLSLQSSEKSSLQTMLNTCSY

SEQ ID NO: 8 - protein, 182 aa, Bacillus sp-16840
LPPGTPSKSQAQSQLNALTVKAEDPMTGYSRNLFPHWSSQGNGCNTRQLVLQRDADYYSGNCPVTSGRWYSYFDGVVVTSPSEIDIDHIVPLAEAWRSGASSWTTEKRREFANDLNGPQLIAVTASVNRSKGDQDPSTWQPPRVAARCGYAKWWINTKYRWDLSLQSSEKSSLQTMLNTCSY

SEQ ID NO: 9 - protein, 182 aa, Bacillus sp-62668
LPPGTPSKSEAQSQLTSLTVKPEDPMTGYSRDHFPHWISQGNGCNTRQIVLQRDADYYSGNCPVTTGKWYSYFDGVIVYSPSEIDIDHIVPLAEAWRSGASSWTAEQRRNFANDLNGPQLIAVTASVNRSKGDQDPSTWQPPRTGARCAYAKWWINTKYRWGLHLQSSEKSSLQSMLNGCAY

SEQ ID NO: 10 - protein, 183 aa, Bacillus sp-13395
AFPPGTPSKSTAQSQLNSLTVKSEGSMTGYSRDKFPHWISQGDGCDTRQLVLKRDGDYYSGNCPVTSGKWYSYYDGIAVYSPSEIDIDHIVPLAEAWRSGASGWTTEKRQNFANDLNGPQLIAVTASVNRSKGDQDPSTWQPPRSGSHCAYAKMWVNTKYRWGLHLQSAEKSALQSMLNACSY

SEQ ID NO: 11 - protein, 185 aa, Bacillus horneckiae
ASAFPPGTPSKSTAQSQLNSLTVKSEGSMTGYSRDKFPHWISQGDGCDTRQLVLKRDGDYYSGNCPVTSGKWYSYYDGITVYSPSEIDIDHIVPLAEAWRSGASGWTTEKRQSFANDLNGPQLIAVTASVNRSKGDQDPSTWQPPRSGSHCAYAKMWVNTKYRWGLHVQSAEKSALQSMLNACSY

SEQ ID NO: 12 - protein, 182 aa, Bacillus sp-11238
FPPEIPSKSTAQSQLNSLTVKSEDAMTGYSRDKFPHWISQGDGCDTRQMVLKRDADYYSGSCPVTSGKWYSYYDGITVYSPSEIDIDHIVPLAEAWRSGASSWTTEKRRNFANDLNGPQLIAVTASVNRSKGDQDPSTWQPPRSGARCAYAKMWVNTKYRWGLHLQSAEKSGLESMLNTCSY

SEQ ID NO: 13 - protein, 182 aa, Bacillus cibi [sequence omitted]

SEQ ID NO: 14 - protein, 182 aa, Bacillus sp-18318
FPPGTPSKSTAQSQLNSLTVKSEGSMTGYSRDKFPHWIGQGSGCDTRQLVLQRDADYYSGSCPVTSGKWYSYYDGVTFYDPSDLDIDHVVPLAEAWRSGASSWSTQKRKDFANDLSGPQLIAVSASSNRSKGDQDPSTWQPTRSGAACGYSKWWISTKHKWGLSLQSSEKNALQGMLNSCVY

SEQ ID NO: 15 - protein, 182 aa, Bacillus idriensis
LPPGTPSKSTAQSQLNALTVQTEGSMTGYSRDKFPHWISQGNGCDTRQVVLQRDADYYSGTCPVTSGKWYSYYDGVTLYNPSDLDIDHVVALAEAWRSGASSWTTDKREDFANDLSGTQLIAVSASTNRSKGDQDPSTWQPPRSGAACGYAKWWISTKYKWNLNLQSSEKTALQSMLNSCSY

SEQ ID NO: 16 - protein, 182 aa, Bacillus algicola
FPPGTPSKSEAQSQLNSLTVQSEGSMSGYSRDKFPHWIGQGNGCDTRQLVLQRDADYYSGDCPVTSGKWYSYFDGVTVYDPSDLDIDHMVPMAEAWRSGASSWSTQKREDFANDLSGPHLIAVTASSNRSKGDQDPSTWKPTRYGAHCGYAKWWINTKYVYDLTLQSSEKTELQSMLNTCSY

SEQ ID NO: 17 - protein, 182 aa, Enviromental sample J
LPPNIPSKADALTKLNALTVQTEGPMTGYSRDLFPHWSSQGNGCNTRHVVLKRDADSVVDTCPVTTGRWYSYYDGLVFTSASDIDIDHVVPLAEAWRSGASSWTSTKRQSFANDLNGPQLIAVSATSNRSKGDQDPSTWQPPRAGARCAYAKMWVETKSRWGLTLQSSEKAALQTAINACSY

SEQ ID NO: 18 - protein, 182 aa, Bacillus vietnamensis
FPPGTPSKSTAQSQLNALTVKSESSMTGYSRDKFPHWIGQRNGCDTRQLVLQRDADSYSGSCPVTSGSWYSYYDGVTFTDPSDLDIDHVVPLAEAWRSGASSWTTAKREDFANDLSGPQLIAVSASSNRSKGDQDPSTWQPPRSGAACGYSKWWISTKYKWGLSLQSSEKTALQGMLNSCIY

SEQ ID NO: 19 - protein, 182 aa, Bacillus hwajinpoensis
IPPGTPSKSAAQSQLDSLAVQSEGSMSGYSRDKFPHWIGQGNGCDTRQLVLQRDADYYSGDCPVTSGKWYSYFDGVQVYDPSYLDIDHMVPLAEAWRSGASSWSTQKREDFANDLDGPHLIAVTASSNRSKGDQDPSTWKPTRYSAHCGYAKWWINTKYVYDLNLQSSEKSALQSMLNTCSY

SEQ ID NO: 20 - protein, 182 aa, Paenibacillus mucilaginosus
LPPGTPSKSTAQSQLNSLTVKSESTMTGYSRDKFPHWTSQGGGCDTRQVVLKRDADYYSGSCPVTSGKWYSYYDGITVYSPSEIDIDHIVPLAEAWRSGASSWTTEKRQNFANDLGGPQLIAVTASSNRAKGDQDPSTWKPTRSGAHCAYAKWWINTKYRWGLHLQSSEKTALQSMLNTCSY

SEQ ID NO: 21 - protein, 182 aa, Bacillus indicus
TPPGTPSKSTAQTQLNALTVKTEGSMTGYSRDLFPHWISQGSGCDTRQVVLKRDADYYSGSCPVTSGKWYSYYDGVTFYDPSDLDIDHIVPLAEAWRSGASSWTTSKRQDFANDLSGPQLIAVSASTNRSKGDQDPSTWQPPRAGAACGYSKWWISTKYKWGLSLQSSEKTALQGMLNSCSY

SEQ ID NO: 22 - protein, 182 aa, Bacillus marisflavi
TPPVTPSKATSQSQLNGLTVKTEGAMTGYSRDKFPHWSSQGGGCDTRQVVLKRDADSYSGNCPVTSGSWYSYYDGVKFTNPSDLDIDHIVPLAEAWRSGASSWTTAQREAFANDLSGSQLIAVSASSNRSKGDQDPSTWQPPRAGAKCGYAKWWISTKSKWNLSLQSSEKTALQGMLNSCVY

SEQ ID NO: 23 - protein, 184 aa, Bacillus luciferensis
ASLPPGIPSLSTAQSQLNSLTVKSEGSLTGYSRDVFPHWISQGSGCDTRQVVLKRDADYYSGNCPVTSGKWYSYYDGVTVYSPSEIDIDHVVPLAEAWRSGASSWTTEKRQNFANDLNGPQLIAVTASSNRSKGDQDPSTWQPTRTGARCAYAKMWINTKYRWGLHLQSSEKSALQSMLNTCSY

SEQ ID NO: 24 - protein, 182 aa, Bacillus marisflavi
TPPVTPSKETSQSQLNGLTVKTEGAMTGYSRDKFPHWSSQGGGCDTRQVVLKRDADSYSGNCPVTSGSWYSYYDGVKFTHPSDLDIDHIVPLAEAWRSGASSWTTAQREAFANDLSGSQLIAVSASSNRSKGDQDPSTWQPPRAGAKCGYAKWWISTKSKWNLSLQSSEKTALQGMLNSCVY

SEQ ID NO: 25 - protein, 182 aa, Bacillus sp. SA2-6
LPSGIPSKSTAQSQLNSLTVKSEGSMTGYSRDKFPHWISQGGGCDTRQVVLKRDADYYSGNCPVTSGKWYSYYDGISVYSPSEIDIDHVVPLAEAWRSGASSWTTTKRQNFANDLNGPQLIAVTASVNRSKGDQDPSTWQPPRYGARCAYAKMWINTKYRWDLNLQSSEKSSLQSMLDTCSY

SEQ ID NO: 26 - protein, 191 aa, Pyrenochaetopsis sp.
LPSPLLIARSPPNIPSATTAKTQLAGLTVAPQGPQTGYSRDLFPHWITQSGTCNTREVVLKRDGTNVVTNSACASTSGSWLSPYDGKTWDSASDIQIDHLVPLSNAWKSGAAAWTTAQRQAFANDLTHPQLVAVTGSVNESKGDDGPEDWKPPLASYYCTYASMWTAVKSNYKLTITSAEKSALTSMLATC

SEQ ID NO: 27 - protein, 190 aa, Vibrissea flavovirens
TPLPIIARTPPNIPTTATAKSQLAALTVAAAGPQTGYSRDLFPTWITISGTCNTRETVLKRDGTNVVVDSACVATSGSWYSPYDGATWTAASDVDIDHMVPLSNAWKSGASAWTTAQRQTFANDLTNPQLLAVTDNVNQAKGDSGPEDWKPSLTSYWCTYAKMWVKVKTVYDLTITSAEKTALTTMLNTC

SEQ ID NO: 28 - protein, 192 aa, Setosphaeria rostrata
APTSSPLVARAPPNVPSKAEATSQLAGLTVAPQGPQTGYSRDLFPHWITQSGTCNTRETVLKRDGTNVVTNSACASTSGSWFSPYDGATWTAASDVDIDHMVPLSNAWKSGAASWTTARRQAFANDLTNPQLLAVTDNVNQAKGDKGPEDWKPPLTSYYCTYSKMWIKVKSVWGLTITSAEKSALTSMLATC

SEQ ID NO: 29 - protein, 192 aa, Endophragmiella valdina
APVPGHLMPRAPPNVPTTAAAKTALAGLTVQAQGSQTGYSRDLFPHWITQSGTCNTREVVLKRDGTNVVTDSACAATSGTWVSPYDGATWTAASDVDIDHMVPLSNAWKSGAASWTTAQRQAFANDLTNPQLLAVTDNVNQSKGDKGPEDWKPPLTSYYCTYAKMWVKVKSVYSLTITSAEKTALTSMLNTC

SEQ ID NO: 30 - protein, 190 aa, Corynespora cassiicola
LPAPLVPRAPPGIPTTSAARSQLAGLTVAAQGPQTGYSRDLFPHWITQSGSCNTREVVLARDGTGVVQDSSCAATSGTWRSPFDGATWTAASDVDIDHMVPLSNAWKSGAASWTTSRRQAFANDLTNPQLIAVTDNVNQSKGDKGPEDWKPPLTSYYCTYAKMWVRVKSVYSLTITSAEKSALTSMLDTC

SEQ ID NO: 31 - protein, 192 aa, Paraphoma sp. XZ1965
APAPVHLVARAPPNVPTAAQAQTQLAGLTVAAQGPQTGYSRDLFPHWITQSGACNTRETVLKRDGTGVVQDSACAATSGTWKSPYDGATWTAASDVDIDHMVPLSNAWKSGAASWTTARRQAFANDLTNPQLLAVTDNVNQAKGDKGPEDWKPPLTSYYCIYARMWIKVKSVYSLTITSAEKSALTSMLGTC

SEQ ID NO: 32 - protein, 186 aa, Monilinia fructicola
TPVPAPTGIPSTSVANTQLAALTVAAAGSQDGYSRDLFPHWITISGACNTRETVLKRDGTNVVVNSACAATSGTWVSPYDGATWTAASDVDIDHLVPLSNAWKAGASSWTTAQRQAFANDLVNPQLLAVTDSVNQGKSDSGPEAWKPSLKSYWCTYAKMWIKVKYVYDLTITSAEKSALVTMMDTC

SEQ ID NO: 33 - protein, 190 aa, Curvularia lunata
APAPLSARAPPNIPSKADATSQLAGLTVAAQGPQTGYSRDLFPHWITQSGTCNTRETVLKRDGTNVVTSSSCAATSGTWFSPYDGATWTAASDVDIDHVVPLSNAWKSGAASWTTARRQAFANDLTNPQLIAVTDSVNQAKGDKGPEDWKPPLSSYYCTYSKMWIKVKSVYGLTVTSAEKSALSSMLATC

SEQ ID NO: 34 - protein, 191 aa, Penicillium reticulisporum
LPAPEALPAPPGVPSASTAQSELAALTVAAQGSQDGYSRSKFPHWITQSGSCDTRDVVLKRDGTNVVQSASGCTITSGKWVSPYDGATWTASSDVDIDHLVPLSNAWKSGASGWTTAARQAFANDLTNPQLLVVTDNVNESKGDKGPEEWKPPLTSYYCTYAEMWVKVKSVYKLTITSAEKSALTSMLSTC

SEQ ID NO: 35 - protein, 191 aa, Penicillium quercetorum
LPAPEPAPSPPGIPSASTARSELASLTVAPQGSQDGYSRAKFPHWIKQSGSCDTRDVVLERDGTNVVQSSTGCTITGGTWVSPYDGATWTASSDVDIDHLVPLSNAWKSGASAWTTAQRQAFANDLTNPQLVAVTDNVNEAKGDKGPEEWKPPLTSYYCTYAEMWVKVKSVYKLTITSAEKSALSSMLNTC

SEQ ID NO: 36 - protein, 192 aa, Setophaeosphaeria sp.
LPAPVTLEARAPPNIPSTASANTLLAGLTVAAQGSQTGYSRDLFPHWITQSGTCNTRETVLKRDGTGVVTDSACASTSGSWYSVYDGATWTAASDVDIDHVVPLSNAWKSGAASWTTARRQSFANDLTNPQLIAVTDNVNQAKGDKGPEDWKPPLTSYYCTYAKMWVKVKSVYSLTITSAEKTALTSMLNTC

SEQ ID NO: 37 - protein, 192 aa, Alternaria sp. XZ2545
LPAPVTLEARAPPNIPTTAAAKTQLAGLTVAAQGPQTGYSRDLFPHWITQSGTCNTRETVLKRDGTGVVTDSACASTSGSWFSVYDGATWTAASDVDIDHVVPLSNAWKSGAASWTTARRQSFANDLTNPQLIAVTDNVNQAKGDKGPEDWKPPLTSYYCTYAKMWVKVKSVYALTITSAEKTALTSMLNTC

SEQ ID NO: 38 - protein, 192 aa, Alternaria sp.
LPAPVTLEARAPPNIPTTAAAKTQLAGLTVAAQGPQTGYSRDLFPHWITQSGSCNTREVVLQRDGTGVVTDSACAATSGSWYSVYDGATWTAASDVDIDHMVPLSNAWKSGAASWTTARRQAFANDLTNPQLLAVTDNVNQAKGDKGPEDWKPPLTSYYCTYAKMWVKVKSVYALTITSAEKTALTSMLNTC

SEQ ID NO: 39 - protein, 186 aa, Trichoderma reesei
APLPAPPGIPSEDTARTQLAGLTVAVVGSGTGYSRDLFPTWDAISGNCNAREYVLKRDGEGVQVNNACEAQSGSWISPYDNASFTNASSLDIDHMVPLKNAWISGASTWTTAQREALANDVSRPQLWAVSASSNRSKGDRSPDQWKPPLTSFYCTYAKSWIDVKSYYKLTITSAEKTALSSMLDTC

SEQ ID NO: 40 - protein, 188 aa, Chaetomium thermophilum
APAPQPTPPGIPSRSTAQSYLNSLTVAASYDDGNYNRDLFPHWNTVSGTCNTREYVLKRDGSNVVTNSACQATSGTWYSPYDGATWTAASDIDIDHMVPLKNAWISGANTWSSSKRSSFANDINSPQLWAVTDSVNQSKGDKSPDKWKPPLTTFYCTYAKSWITVKYNYNLTITSAEKSALQNMINTC

SEQ ID NO: 41 - protein, 190 aa, Scytalidium thermophilum
LPAPAPMPTPPGIPSKSTAQSQLNALTVKASYDDGKYKRDLFPHWNTVSGTCNTREYVLKRDGVNVVTNSACAATSGTWYSPFDGATWTAASDVDIDHMVPLKNAWISGANNWTSTKRTQFANDINLPQLWAVTDDVNQAKGDKSPDKWKPPLTSFYCTYAKSWITVKYNYGLSITSAEKSALTSMINTC

SEQ ID NO: 42 - protein, 186 aa, Metapochonia suchlasporia
VPVPAPPGIPSTSTAKTLLAGLKVAVPLSGDGYSREKFPLWETIQGTCNAREFVLKRDGTDVKTNNACVAESGNWVSPYDGVKFTAARDLDIDHMVPLKNAWISGASQWTTERRKALANDITRPQLWAVSAHANRGKSDDSPDEWKPPLKTFWCTYAKSWVQVKSFYELTITDAEKGALAGMLDSC

SEQ ID NO: 43 - protein, 198 aa, Daldinia fissa
APAPIPVAEPAPMPMPTPPGIPSASSAKSQLASLTVKAAVDDGGYQRDLFPTWDTITGTCNTREYVLKRDGANVQVGSDCYPTSGTWTSPYDGGKWTSPSDVDIDHMVPLKNAWVSGANKWTTAKREQFANDVDRPQLWAVTDNVNSSKGDKSPDTWKPPLTSFYCTYASAYVAVKSYWGLTITSAEKSALSDMLGTC

SEQ ID NO: 44 - protein, 188 aa, Acremonium sp. XZ2007
LPLQSRDPPGIPSTATAKSLLNGLTVKAWSNEGTYDRDLFPHWQTIEGTCNAREYVLKRDGQNVVVNSACTAQSGTWKSVYDGETTNSASDLDIDHMIPLKNAWISGAATWTTAQRTSFANDISSPQLWAVTAGVNRSKSDRSPDTWVPPLASFHCTYGKAWVQVKSKWALSITSAEKSALTGLLNKC

SEQ ID NO: 45 - protein, 182 aa, Acremonium dichromosporum
IPPGIPSEATARSLLSSLTVAPTVDDGTYDRDLFPHWSSVEGNCNAREFVLRRDGDGVSVGNDCYPTAGTWTCPYDGKRHSVPSDVSIDHMVPLHNAWMTGASEWTTAEREAFANDIDGPQLWAVTSTTNSQKGSDAPDEWQPPQTSIHCKYAAAWIQVKSTYDLTVSSAEQAALEEMLGRC

SEQ ID NO: 46 - protein, 188 aa, Sarocladium sp. XZ2014
VPIPLPDPPGIPSSSTANTLLAGLTVRASSNEDTYNRDLFPHWVAISGNCNAREYVLRRDGTNVVVNTACVPQSGTWRSPYDGESTTNASDLDIDHMVPLKNAWISGAASWTTAKRQDFANDVSGPQLWAVTAGVNRSKGDKSPDSWVPPLASFHCTYARSWIQVKSSWALSVTSAEKAALTDLLSTC

SEQ ID NO: 47 - protein, 186 aa, Metarhizium sp. HNA15-2
VPVPAPPGIPTASTARTLLAGLKVATPLSGDGYSRTLFPTWETIEGTCNAREFVLKRDGTDVQTNTACVAQSGNWVSPYDGVAFTAASDLDIDHMVPLKNAWISGASQWTTDKRKGLANDITRPQLWAVSAHANRAKGDSSPDEWKPPLKTFWCTYARSWVQVKSYYALTITDAEKGALSGMLDSC

SEQ ID NO: 48 - protein, 188 aa, Acremonium sp. XZ2414
APIAVRDPPGIPSASTANTLLAGLTVRASSNEDSYDRNLFPHWSAISGNCNAREFVLERDGTNVVVNNACVAQSGTWRSPYDGETTGNASDLDIDHMVPLKNAWISGASSWSTTRRQEFANDVSGPQLWAVTAGVNRSKGDRSPDSWVPPLASFHCTYAKSWVQVKSSWSLSVTSAEKAALSDLLGTC

SEQ ID NO: 49 - protein, 186 aa, Isaria tenuipes
APVPEPPGIPSTSTAQSDLNSLQVAASGSGDGYSRAEFPHWVSVEGSCDSREYVLKRDGQDVQADSSCKITSGTWVSPYDATTWTNSSKVDIDHLVPLKNAWISGASSWTKAQRQDFANDIKRPQLYAVSENANRSKGDRSPDGWKPPLKSFYCTYAKSWVAVKSYYKLTITSAEKSALGDMLDTC

SEQ ID NO: 50 - protein, 184 aa, Scytalidium circinatum
APPGIPSASTASSLLGELAVAEPVDDGSYDRDLFPHWEPIPGETACSAREYVLRRDGTGVETGSDCYPTSGTWSSPYDGGSWTAPSDVDIDHMVPLKNAWISGASEWTTAEREAFANDIDGPQLWAVTDEVNQSKSDQSPDEWKPPLSSFYCTYACAWIQVKSTYSLSISSAEQAALEDMLGSC

SEQ ID NO: 51 - protein, 186 aa, Metarhizium lepidiotae
VPVPAPPGIPTASTARTLLAGLKVATPLSGDGYSRTLFPTWETIEGTCNAREFVLKRDGTDVQTNTACVAESGNWVSPYDGVSFTAASDLDIDHMVPLKNAWISGASQWTTDKRKDLANDITRPQLWAVSAHANRSKGDSSPDEWKPPLQTFWCTYSKSWIQVKSHYSLTITDAEKGALSGMLDSC

SEQ ID NO: 52 - protein, 226 aa, Thermobispora bispora
LDIADGRPAGGKAAEAATGTSPLANPDGTRPGLAAITSADERAEARALIERLRTKGRGPKTGYEREKFGYAWADSVDGIPFGRNGCDTRNDVLKRDGQRLQFRSGSDCVVISMTLFDPYTGKTIEWTKQNAAEVQIDHVVPLSYSWQMGASRWSDEKRRQLANDPLNLMPVDGATNSRKGDSGPASWLPPRREIRCAYVVRFAQVALKYDLPVTTADKETMLQQCS

SEQ ID NO: 53 - protein, 191 aa, Sporormia fimetaria
LPAPVLEKRTPPNIPSTSTAQSLLSGLTVAPQGSQTGYSRDLFPHWITVSGTCNTRETVLKRDGSNVVTDSACASVSGSWYSTYDGATWTAASDVDIDHVVPLSNAWKSGAASWTTARRQAFANDLTNPQLIAVTDNVNQAKGDQGPESWKPPLTSYYCTYAKMWVKVKSVYSLTVTSAEKSALSSMLGTC

SEQ ID NO: 54 - protein, 193 aa, Pycnidiophora cf.dispera
LPAPAPVLVAREPPNIPSTSSAQSMLSGLTVKAQGPQDGYSRDLFPHWITISGTCNTRETVLKRDGTNVVTNSACASTSGSWYSPYDGATWTAASDVDIDHIVPLSNAWKSGAASWTTSRRQQFANDLTNPQLIAVTDSVNQAKGDKGPEDWKPSRTSYHCTYAKMWIKVKSVYSLTVTSAEKSALTTMLNTC

SEQ ID NO: 55 - protein, 199 aa, Enviromental sample D
DTDPEPVAGSALEALAGLEVKGPGPDTGYERALFGPPWADVDGNGCDTRNDILARDLTDLTFSTRGDVCEVRTGTFDDPYTGETIDFRRGNATSAAVQIDHVVPLLDAWRKGARAWDDETRRQFANDPLNLLASDGPANQSKGARDASAWLPPNHAFRCPYVARQIAVKAAYELSVTPSESEAMARVLADCPAEPLPAG

SEQ ID NO: 56 - protein, 199 aa, Enviromental sample O
DDEPEPARGSALEALARLEVVGPGPDTGYERELFGPAWADVDGNGCDTRNDILARDLTDLTFSTRGEVCEVRTGTFQDPYTGETIDFRRGNATSMAVQIDHVVPLMDAWRKGARAWDDETRRQFANDPLNLLASDGPANQSKGARDASAWLPPNHAFRCPYVARQIAVKTAYELSVTPSESEAMARVLEDCPAEPVPAG

SEQ ID NO: 57 - protein, 186 aa, Clavicipitaceae sp-70249
VPVPAPPGIPSTSTAKTLLAGLKVATPLSGDGYSRDKFPTWETIQGTCNAREFVIKRDGTDVKTNSACVAESGNWVSPYDGVKFTAARDLDIDHMVPLKNAWISGASQWTTEQRKALANDITRPQLWAVSAHANRGKSDDSPDEWKPPLKTFWCTYAKSWVQVKSFYKLTITDTEKGALAGMLDTC

SEQ ID NO: 58 - protein, 187 aa, Westerdykella sp. AS85-2
FPAPASVLEARAPPNIPSASTAQSLLVGLTVQPQGPQDGYSRDLFPHWITISGTCNTRETVLKRDGSNVVTNSACAATSGTWYSPYDGATWTSASDVDIDHLVPLSNAWKSGAASWTTAKRQQFANDLTNPQLLAVTDRVNQAKGDKGPEAWKPSLASYHCTYAKMWVKVKSKDVRLTGNWTKDDGW

SEQ ID NO: 59 - protein, 194 aa, Humicolopsis cephalosporioides
APTPAPVELERRTPPNIPTTASAKSLLAGLTVAAQGPQTGYSRDLFPHWITISGSCNTRETVLKRDGTGVVTDSACASTAGSWYSPYDGATWTAASDVDIDHMVPLSNAWKSGAAQWTTARRQDFANDLTNPQLFAVTDNVNQEKGDKGPEDWKPSLTSYYCTYAKAWVKVKSVWALTITSAEKSALTTMLNTC

SEQ ID NO: 60 - protein, 190 aa, Neosartorya massa
IPAPVALPTPPGIPSAATAESELAALTVAAQGSSSGYSRDLFPHWISQGGSCNTREVVLARDGSGVVKDSNCYPTSGSWYSPYDGATWTQASDVDIDHVVPLANAWRSGASKWTTSQRQAFANDLTNPQLMAVTDNVNQAKGDDGPEAWKPPLTSYYCTYAKMWVRVKYVYDLTITSAEKSALVSMLDTC

SEQ ID NO: 61 - protein, 191 aa, Roussoella intermedia
APTPALLPRAPPNIPSTATAKSQLAALTVAAQGPQDGYSRDLFPHWITQSGSCNTREVVLKRDGTNVVQDSSCAATSGTWVSPFDGATWTAASDVDIDHLVPLSNAWKSGAASWTTARRQSFANDLTNPQLLAVTDEVNQAKGDKGPEAWKPPLASYHCTYAKMWVKVKSTYSLTITSAEKSALTTMLNTC

SEQ ID NO: 62 - protein, 191 aa, Pleosporales
LPTPSLVKRTPPNIPSTTSAKSLLAGLTVAAQGPQDGYSRDLFPHWITISGTCNTRETVLKRDGTNVVTDSACASTSGSWYSTYDGATWTAASDVDIDHVVPLSNAWKSGAASWTTARRQSFANDLTNPQLIAVTDSVNQSKGDKGPESWKPPLTSYHCTYAKMWVKVKDVYSLTVTSAEKSALTTMLNTC

SEQ ID NO: 63 - protein, 192 aa, Phaeosphaeria sp.
LPAPIHLTARAPPNIPSASEARTQLAGLTVAAQGPQDGYSRDLFPHWITQSGTCNTRETVLKRDGTNVVTNSACASTSGSWFSPYDGATWTAASDVDIDHMVPLSNAWKSGAASWTTARRQAFANDLTNPQLLAVTDNVNQAKGDKGPEDWKPPLTSYYCTYARMWVKVKSVYALTVTSAEKSALTSMLGTC

SEQ ID NO: 64 - protein, 189 aa, Didymosphaeria futilis
LPTPNTLEARAPPNIPSTSAAQSQLSALTVAAQGPQTGYSRDLFPHWITQSGTCNTRETVLKRDGTNVLTDSACASTSGSWKSPYDGATWTAASDVDIDHVVPLSNAWKSGAASWTTARRQSFANDLTNPQLIAVTDNVNQAKGDKGPEDWKPPLTSYYCTYAKMWVKVKSVYSLTITSAEKSALTMLA

SEQ ID NO: 65 - protein, 109 aa, Bacillus licheniformis
ARYDDILYFPASRYPETGAHISDAIKAGHSDVCTIERSGADKRRQESLKGIPTKPGFDRDEWPMAMCEEGGKGASVRYVSSSDNRGAGSWVGNRLSGFADGTRILFIVQ

SEQ ID NO: 66 - protein, 110 aa, Bacillus subtilis
ASSYDKVLYFPLSRYPETGSHIRDAIAEGHPDICTIDRDGADKRREESLKGIPTKPGYDRDEWPMAVCEEGGAGADVRYVTPSDNRGAGSWVGNQMSSYPDGTRVLFIVQ

SEQ ID NO: 67 - protein, 221 aa, Aspergillus oryzae
VPVNPEPDATSVENVALKTGSGDSQSDPIKADLEVKGQSALPFDVDCWAILCKGAPNVLQRVNEKTKNSNRDRSGANKGPFKDPQKWGIKALPPKNPSWSAQDFKSPEEYAFASSLQGGTNAILAPVNLASQNSQGGVLNGFYSANKVAQFDPSKPQQTKGTWFQITKFTGAAGPYCKALGSNDKSVCDKNKNIAGDWGFDPAKWAYQYDEKNNKFNYVGK

SEQ ID NO: 68 - protein, 188 aa, Trichoderma harzianum
APAPMPTPPGIPTESSARTQLAGLTVAVAGSGTGYSRDLFPTWDAISGNCNAREYVLKRDGEGVQVNNACESQSGTWISPYDNASFTNASSLDIDHMVPLKNAWISGASSWTTAQREALANDVSRPQLWAVSASANRSKGDRSPDQWKPPLTSFYCTYAKSWIDVKSFYKLTITSAEKTALSSMLDTC

SEQ ID NO: 69 - protein, 5 aa, Artificial
  Motif
  MISC_FEATURE (1)..(1): Xaa = Thr (T) or Asp (D) or Ser (S)
  MISC_FEATURE (2)..(2): Xaa = Gly (G) or Asn (N)
XXPQL

SEQ ID NO: 70 - protein, 5 aa, Artificial
  Motif
  MISC_FEATURE (1)..(1): Xaa = F (phe) or L (Leu) or Y (Tyr) or I (Ile)
  MISC_FEATURE (3)..(3): Xaa = N (Asn) or R (Arg)
  MISC_FEATURE (5)..(5): Xaa = L (Leu) or I (Ile) or P (Phe) or V (Val)
XAXDX

SEQ ID NO: 71 - protein, 4 aa, Artificial
  Motif
  MISC_FEATURE (2)..(2): Xaa= Asp (D) or Asn (N)
  MISC_FEATURE (4)..(4): Xaa= Ala (A) or Arg (R)
CXTX

SEQ ID NO: 72 - protein, 4 aa, Artificial
  Motif
  MISC_FEATURE (1)..(1): Xaa = Asp (D) or Gln (Q)
  MISC_FEATURE (2)..(2): Xaa = Ile (I) or Val (V)
XXDH

SEQ ID NO: 73 - protein, 7 aa, Artificial
  Motif
  MISC_FEATURE (1)..(1): Xaa = Asp (D) or Met (M) or Leu (L)
  MISC_FEATURE (2)..(2): Xaa = Ser (S) or Thr (T)
  MISC_FEATURE (7)..(7): Xaa = Asp (D) or Asn (N)
XXGYSRX

SEQ ID NO: 74 - protein, 8 aa, Artificial
  Motif
  MISC_FEATURE (3)..(3): Xaa = any amino acid
ASXNRSKG

SEQ ID NO: 75 - protein, 8 aa, Artificial
  Motif
  MISC_FEATURE (1)..(1): Xaa = Val (V) or Ile (I)
  MISC_FEATURE (4)..(4): Xaa = Ser (S) or Ala (A)
XPLXNAWK

SEQ ID NO: 76 - protein, 4 aa, Artificial
  Motif
NPQL

SEQ ID NO: 77 - protein, 4 aa, Artificial
  Motif
  MISC_FEATURE (2)..(2): Xaa = Gln (Q) or Glu(E)
  MISC_FEATURE (4)..(4): Xaa = Trp (W) or Tyr (Y)
PXLX

SEQ ID NO: 78 - protein, 4 aa, Artificial
  Motif
  MISC_FEATURE (1)..(1): Xaa=Lys (K) or His (H) or Glu (E)
XNAW

SEQ ID NO: 79 - protein, 269 aa, Bacillus lentus
AQSVPWGISRVQAPAAHNRGLTGSGVKVAVLDTGISTHPDLNIRGGASFVPGEPSTQDGNGHGTHVAGTIAALNNSIGVLGVAPSAELYAVKVLGASGSGSVSSIAQGLEWAGNNGMHVANLSLGSPSPSATLEQAVNSATSRGVLVVAASGNSGAGSISYPARYANAMAVGATDQNNNRASFSQYGAGLDIVAPGVNVQSTYPGSTYASLNGTSMATPHVAGAAALVKQKNPSWSNVQIRNHLKNTATSLGSTNLYGSGLVNAEAATR

SEQ ID NO: 80 - protein, 275 aa, Bacillus amyloliquefaciens [sequence omitted]

SEQ ID NO: 81 - protein, 311 aa, Bacillus sp. [sequence omitted]

SEQ ID NO: 82 - protein, 269 aa, Bacillus lentus
AQSVPWGIERVQAPAAHNRGLTGSGVKVAVLDTGISTHPDLRIRGGASFVPGEPSTQDGNGHGTHVAGTIAALDNSIGVLGVAPSAELYAVKVLGASGSGSVSSIAQGLEWAGNNGMHVANLSLGSPSPSATLEQAVNSATSRGVLVVAASGNSGAGSISYPARYANAMAVGATDQNNNRASFSQYGAGLDIVAPGVNILSTWPGSTYASLNGTSMATPHVAGAAALVKQKNPSWSNVQIRNHLKNTATSLGDTWEYGSGLVNAEAATR

SEQ ID NO: 83 - protein, 311 aa, Bacillus sp.
AVPSTQTPWGIKSIYNDQSITKTTGGKGIKVAVLDTGVYTSHLDLAGSAEQCKDFTQSNPLVDGSCTDRQGHGTHVAGTVLAHGGSNGQGVYGVAPQAKLWAYKVLGDKGEGYSDDIAAAIRHVADEASRTGSKVVINMSLGSSAKDSLIASAVDYAYGKGVLIVAAAGNEGPKPNTIGYPAGFVNAVAVAALENVQEKGTYRVADFSSRGNPATAGDYIIQERDIEVSAPGASVESTWYTGGYNTISGTSMATPHVAGLAAKIWSANTSLSHSQLRTELQNRAKVYDIKGGIGAGPGDDYASGFGYPRVK

SEQ ID NO: 84 - protein, 269 aa, Bacillus lentus
AQTIPWGISRVQAPAAHNRGLTGSGVKVAVLDTGISTHPDLNIRGGASFVPGEPSTQDGNGHGTHVAGTIAALNNSIGVLGVAPSAELYAVKVLGADGEGAISSIAQGLEWAGNNGMHVANLSLGSPSPSATLEQAVNSATSRGVLVVAASGNSGASSISYPARYANAMAVGATDQNNNRASFSQYGAGLDIVAPGVNIQSTYPGSTYASLNGTSMATPHVAGAAALVKQKNPSWSNVQIRNHLKNTATSLGSTNLYGSGLVNAEAATR

SEQ ID NO: 85 - protein, 269 aa, Bacillus lentus
AQSVPWGISRVQAPAAHNRGLAGSGVKVAVLDTGISTHPDLNIRGGASFVPGEPSTQDGDGHGTHVAGTIAALNNSIGVLGVAPSAELYAVKVLGASGGGAISSIAQGLEWAGLNGMHVANLSLGSPSPSATLEQAVNSATSRGVLVVAASGNSGADSISYPARYANAMAVGATDQNNNRADFSQYGAGLDIVAPGVNVQSTYPGSAYASLNGTSMATPHVAGAAVLVKQKNPSWSNVRIRDHLKNTATSLGSTNLYGSGLVNAFAATR

SEQ ID NO: 86 - protein, 269 aa, Bacillus lentus
AQSVPWGISRVQAPAAHNRGLRGSGVKVAVLDTGISTHPDLNIRGGASFVPGEPSTQDGNGHGTHVAGTIAALNNSIGVLGVAPSAELYAVKVLGASGGGAISSIAQGLEWAGNNGMHVANLSLGSPSPSATLEQAVNSATSRGVLVVAASGNSGAGSISYPARYANAMAVGATDQNNNRASFSQYGAGLDIVAPGVNVQSTYPGSTYASLNGTSMATPHVAGAAVLVKQKNPSWSNVRIRNHLKNTATSLGSTNLYGSGLVNAEAATR